European Patent Specification EP 3 795 677 B1, published February 11, 2026. Title: A composition for stimulating differentiation of stem cell comprising multi-layer graphene film and culture broth of progenitor cell. Applicant: Seoul National University R&DB Foundation. The sequence listing filed with the application follows.

SEQUENCE LISTING (16 sequences)

SEQ ID NO: 1 - DNA, 20 bp, Artificial Sequence
  Beta-actin forward primer
atgaagcccagagcaaaaga

SEQ ID NO: 2 - DNA, 20 bp, Artificial Sequence
  Beta-actin reverse primer
ggggtgttgaaggtctcaaa

SEQ ID NO: 3 - DNA, 20 bp, Artificial Sequence
  SOX9 forward primer
gctttctcgcatgaatctcc

SEQ ID NO: 4 - DNA, 20 bp, Artificial Sequence
  SOX9 reverse primer
ttggggaaggtgttctcttg

SEQ ID NO: 5 - DNA, 20 bp, Artificial Sequence
  COLLAGEN TYPE I forward primer
caaaccaggcgaaaggggtc

SEQ ID NO: 6 - DNA, 19 bp, Artificial Sequence
  COLLAGEN TYPE I reverse primer
aatggaccacggcttccaa

SEQ ID NO: 7 - DNA, 20 bp, Artificial Sequence
  COLLAGEN TYPE II forward primer
aagatgttgtaggaccccga

SEQ ID NO: 8 - DNA, 20 bp, Artificial Sequence
  COLLAGEN TYPE II reverse primer
catctgcgccgcaaagtttc

SEQ ID NO: 9 - DNA, 20 bp, Artificial Sequence
  RUNX2 forward primer
cagaccagcagcactccata

SEQ ID NO: 10 - DNA, 20 bp, Artificial Sequence
  RUNX2 reverse primer
ttgggcaagtttgggtttag

SEQ ID NO: 11 - DNA, 20 bp, Artificial Sequence
  HUMAN GAPDH forward primer
gagtcaacggatttggtcgt

SEQ ID NO: 12 - DNA, 20 bp, Artificial Sequence
  HUMAN GAPDH reverse primer
ttgattttggagggatctcg

SEQ ID NO: 13 - DNA, 19 bp, Artificial Sequence
  HUMAN RUNX2 forward primer
gacagccccaacttcctgt

SEQ ID NO: 14 - DNA, 20 bp, Artificial Sequence
  HUMAN RUNX2 reverse primer
ccggagctcagcagaataat

SEQ ID NO: 15 - DNA, 20 bp, Artificial Sequence
  HUMAN OSTEOCALCIN forward primer
agcaaaggtgcagcctttgt

SEQ ID NO: 16 - DNA, 18 bp, Artificial Sequence
  HUMAN OSTEOCALCIN reverse primer
gcgcctgggtctcttcat